European Patent Specification EP 3 956 445 B1, published July 10, 2024. Title: MULTIPLEX ASSEMBLY OF NUCLEIC ACID MOLECULES. Applicant: Thermo Fisher Scientific GENEART GmbH KUHN, Phillip HOFMEISTER, Thomas PUETZSCHLER, Joern NETUSCHIL, Nikolai KONOVALOVA,Tatiana. Application Unassigned. The sequence listing filed with the application follows.

SEQUENCE LISTING (14 sequences)

SEQ ID NO: 1 - DNA, 34 bp, Artificial Sequence
  Synthetic Primer Sequences
acgtggaagcagagatagacagatagacagataa

SEQ ID NO: 2 - DNA, 31 bp, Artificial Sequence
  Synthetic Primer Sequences
ttcagcagagatagacagatagacagatata

SEQ ID NO: 3 - DNA, 17 bp, Artificial Sequence
  Synthetic Primer Sequences
ctagcccgccccgtatg

SEQ ID NO: 4 - DNA, 17 bp, Artificial Sequence
  Synthetic Primer Sequences
cactgacgcttacgccc

SEQ ID NO: 5 - DNA, 17 bp, Artificial Sequence
  Synthetic Primer Sequences
tcaaaggccgcatcatc

SEQ ID NO: 6 - DNA, 17 bp, Artificial Sequence
  Synthetic Primer Sequences
atagttccttggcgcgg

SEQ ID NO: 7 - DNA, 17 bp, Artificial Sequence
  Synthetic Primer Sequences
tcgggcgagacactacc

SEQ ID NO: 8 - DNA, 17 bp, Artificial Sequence
  Synthetic Primer Sequences
agtgattccgctcccct

SEQ ID NO: 9 - DNA, 17 bp, Artificial Sequence
  Synthetic Primer Sequences
gcgccgcaccattttct

SEQ ID NO: 10 - DNA, 17 bp, Artificial Sequence
  Synthetic Primer Sequences
gtcaatcggtcatcgcc

SEQ ID NO: 11 - DNA, 17 bp, Artificial Sequence
  Synthetic Primer Sequences
cggcccagggagtatta

SEQ ID NO: 12 - DNA, 17 bp, Artificial Sequence
  Synthetic Primer Sequences
acaccgcgagagtcaca

SEQ ID NO: 13 - DNA, 17 bp, Artificial Sequence
  Synthetic Primer Sequences
gcttccgcgacccacta

SEQ ID NO: 14 - DNA, 17 bp, Artificial Sequence
  Synthetic Primer Sequences
agtctgagtgcgccggc